European Patent Application EP 4 317 449 A1, published February 7, 2024. Title: 효소 처리를 통한 2'-푸코실락토오스의 생산성 증대 방법. Applicant: (주)에이피테크놀로지. The sequence listing filed with the application follows.

SEQUENCE LISTING (5 sequences)

SEQ ID NO: 1 - DNA, 1122 bp, Escherichia coli
  source 1..1122: mol_type = genomic DNA
atgtcaaaagtcgctctcatcaccggtgtaaccggacaagacggttcttacctggcagagtttctgctggaaaaaggttacgaggtgcatggtattaagcgtcgcgcatcgtcattcaacaccgagcgcgtggatcacatttatcaggatccgcacacctgcaacccgaaattccatctgcattatggcgacctgagtgatacctctaacctgacgcgcattttgcgtgaagtacagccggatgaagtgtacaacctgggcgcaatgagccacgttgcggtctcttttgagtcaccagaatataccgctgacgtcgacgcgatgggtacgctgcgcctgctggaggcgatccgcttcctcggtctggaaaagaaaactcgtttctatcaggcttccacctctgaactgtatggtctggtgcaggaaattccgcagaaagagaccacgccgttctacccgcgatctccgtatgcggtcgccaaactgtacgcctactggatcaccgttaactaccgtgaatcctacggcatgtacgcctgtaacggaattctcttcaaccatgaatccccgcgccgcggcgaaaccttcgttacccgcaaaatcacccgcgcaatcgccaacatcgcccaggggctggagtcgtgcctgtacctcggcaatatggattccctgcgtgactggggccacgccaaagactacgtaaaaatgcagtggatgatgctgcagcaggaacagccggaagatttcgttatcgcgaccggcgttcagtactccgtgcgtcagttcgtggaaatggcggcagcacagctgggcatcaaactgcgctttgaaggcacgggcgttgaagagaagggcattgtggtttccgtcaccgggcatgacgcgccgggcgttaaaccgggtgatgtgattatcgctgttgacccgcgttacttccgtccggctgaagttgaaacgctgctcggcgacccgaccaaagcgcacgaaaaactgggctggaaaccggaaatcaccctcagagagatggtgtctgaaatggtggctaatgacctcgaagcggcgaaaaaacactctctgctgaaatctcacggctacgacgtggcgatcgcgctggagtcataa

SEQ ID NO: 2 - DNA, 966 bp, Escherichia coli
  source 1..966: mol_type = genomic DNA
atgagtaaacaacgagtttttattgctggtcatcgcgggatggtcggttccgccatcaggcggcagctcgaacagcgcggtgatgtggaactggtattacgcacccgcgacgagctgaacctgctggacagccgcgccgtgcatgatttctttgccagcgaacgtattgaccaggtctatctggcggcggcgaaagtgggcggcattgttgccaacaacacctatccggcggatttcatctaccagaacatgatgattgagagcaacatcattcacgccgcgcatcagaacgacgtgaacaaactgctgtttctcggatcgtcctgcatctacccgaaactggcaaaacagccgatggcagaaagcgagttgttgcagggcacgctggagccgactaacgagccttatgctattgccaaaatcgccgggatcaaactgtgcgaatcatacaaccgccagtacggacgcgattaccgctcagtcatgccgaccaacctgtacgggccacacgacaacttccacccgagtaattcgcatgtgatcccagcattgctgcgtcgcttccacgaggcgacggcacagaatgcgccggacgtggtggtatggggcagcggtacaccgatgcgcgaatttctgcacgtcgatgatatggcggcggcgagcattcatgtcatggagctggcgcatgaagtctggctggagaacacccagccgatgttgtcgcacattaacgtcggcacgggcgttgactgcactatccgcgagctggcgcaaaccatcgccaaagtggtgggttacaaaggccgggtggtttttgatgccagcaaaccggatggcacgccgcgcaaactgctggatgtgacgcgcctgcatcagcttggctggtatcacgaaatctcactggaagcggggcttgccagcacttaccagtggttccttgagaatcaagaccgctttcgggggtaa

SEQ ID NO: 3 - DNA, 1254 bp, Escherichia coli
  source 1..1254: mol_type = genomic DNA
atgtactatttaaaaaacacaaacttttggatgttcggtttattctttttcttttacttttttatcatgggagcctacttcccgtttttcccgatttggctacatgacatcaaccatatcagcaaaagtgatacgggtattatttttgccgctatttctctgttctcgctattattccaaccgctgtttggtctgctttctgacaaactcgggctgcgcaaatacctgctgtggattattaccggcatgttagtgatgtttgcgccgttctttatttttatcttcgggccactgttacaatacaacattttagtaggatcgattgttggtggtatttatctaggcttttgttttaacgccggtgcgccagcagtagaggcatttattgagaaagtcagccgtcgcagtaatttcgaatttggtcgcgcgcggatgtttggctgtgttggctgggcgctgtgtgcctcgattgtcggcatcatgttcaccatcaataatcagtttgttttctggctgggctctggctgtgcactcatcctcgccgttttactctttttcgccaaaacggatgcgccctcttctgccacggttgccaatgcggtaggtgccaaccattcggcatttagccttaagctggcactggaactgttcagacagccaaaactgtggtttttgtcactgtatgttattggcgtttcctgcacctacgatgtttttgaccaacagtttgctaatttctttacttcgttctttgctaccggtgaacagggtacgcgggtatttggctacgtaacgacaatgggcgaattacttaacgcctcgattatgttctttgcgccactgatcattaatcgcatcggtgggaaaaacgccctgctgctggctggcactattatgtctgtacgtattattggctcatcgttcgccacctcagcgctggaagtggttattctgaaaacgctgcatatgtttgaagtaccgttcctgctggtgggctgctttaaatatattaccagccagtttgaagtgcgtttttcagcgacgatttatctggtctgtttctgcttctttaagcaactggcgatgatttttatgtctgtactggcgggcaatatgtatgaaagcatcggtttccagggcgcttatctggtgctgggtctggtggcgctgggcttcaccttaatttccgtgttcacgcttagcggccccggcccgctttccctgctgcgtcgtcaggtgaatgaagtcgcttaa

SEQ ID NO: 4 - DNA, 807 bp, unidentified
  source 1..807: mol_type = genomic DNA
atgatatttgtaaccggatatggccagatgtgtaacaacatccttcaatttgggcatttctttgcttatgcaaaaagaaatggtttaaaaacggttggcttacgtttttgctacaaatacacttttttcaagattagtaacgaaaaaggctataattggccgacctatctttatgcaaaatatggggcaaaaataggacttataaagtctgttgattttgacgaatcattcgaaggtacaaatgtagattctcttcaattagacaaacaaaccgtgttagccaaaggctggtattttagagactaccagggatttcttaattaccgtaatgagcttaaagcacttttcgactttaaagagcatattaagaaaccggtagaacagtttttttcaacgttatcaaaagacaccatcaaagtaggcctgcatataagacgtggtgattataagacctggcaccagggtaaatacttttttagcgacgaagaatacggtcaaatcgtaaattcttttgctaaaagtttagataaaccggtagaattaattattgttagcaatgatcccaaactaaacagcaaaagttttgaaaatttaacatcctgtaaagtatcaatgttaaatggcaatcctgccgaagatctttaccttctttctaaatgtgattatattattggccctcccagcactttttctttaatggcagctttttacgaagaccgccctttatattggatatttgataaagaaaaacagcttttagcagaaaactttgacaagttcgagaatctgtttcgacacattatttaa

SEQ ID NO: 5 - protein, 268 aa, unidentified
MIFVTGYGQMCNNILQFGHFFAYAKRNGLKTVGLRFCYKYTFFKISNEKGYNWPTYLYAKYGAKIGLIKSVDFDESFEGTNVDSLQLDKQTVLAKGWYFRDYQGFLNYRNELKALFDFKEHIKKPVEQFFSTLSKDTIKVGLHIRRGDYKTWHQGKYFFSDEEYGQIVNSFAKSLDKPVELIIVSNDPKLNSKSFENLTSCKVSMLNGNPAEDLYLLSKCDYIIGPPSTFSLMAAFYEDRPLYWIFDKEKQLLAENFDKFENLFRHII